European Patent Specification EP 3 759 241 B1, published February 19, 2025. Title: GENERATION OF SINGLE-STRANDED CIRCULAR DNA TEMPLATES FOR SINGLE MOLECULE SEQUENCING. Applicant: F. Hoffmann-La Roche AG Roche Diagnostics GmbH Roche Sequencing Solutions, Inc. Kapa Biosystems, Inc. The sequence listing filed with the application follows.

SEQUENCE LISTING (7 sequences)

SEQ ID NO: 1 - DNA, 46 bp, Single stranded artificial
atatctctctactgactgtcctcctcctccgtttttgagagatatt

SEQ ID NO: 2 - DNA, 46 bp, Single stranded artificial; identical to SEQ ID NO: 1

SEQ ID NO: 3 - DNA, 46 bp, Single stranded artificial
atatctctcttttcctcctcctccgttgttgttgttgagagatatt

SEQ ID NO: 4 - DNA, 46 bp, Single stranded artificial; identical to SEQ ID NO: 3

SEQ ID NO: 5 - DNA, 36 bp, Single stranded artificial
atctctctctactgactgtcctcctcctccgttttt

SEQ ID NO: 6 - DNA, 60 bp, Single stranded artificial
atctctctcaaatcctcctcctccgttggaggaacggaggaggaggatttgagagagatt

SEQ ID NO: 7 - DNA, 60 bp, Single stranded artificial
atctctctcttttcctcctcctccgttggaggaacggaggaggaggaaaagagagagatt